European Patent Specification EP 3 440 192 B1, published October 2, 2024. Title: Production Of Fully Functional Mature Beta Cells From Human Pancreatic Progenitors. Applicant: The Regents of the University of California. The sequence listing filed with the application follows.

SEQUENCE LISTING (4 sequences)

SEQ ID NO: 1 - DNA, 20 bp, Homo sapiens
  misc_feature: mtDNA 16S rRNA
gccttcccccgtaaatgata

SEQ ID NO: 2 - DNA, 20 bp, Homo sapiens
  misc_feature: mtDNA 16S rRNA
ttatgcgattaccgggctct

SEQ ID NO: 3 - DNA, 25 bp, Homo sapiens
  misc_feature: B2M
tgctgtctccatgtttgatgtatct

SEQ ID NO: 4 - DNA, 22 bp, Homo sapiens
  misc_feature: B2M
tctctgctccccacctctaagt